European Patent Specification EP 3 942 943 B1, published April 24, 2024. Title: Functional food composition and cosmetic composition comprising galacto-oligosaccharide, or galacto-oligosaccharide and collagen tripeptides for improving immune function and skin condition. Applicant: Neo Cremar Co.,Ltd. The sequence listing filed with the application follows.

SEQUENCE LISTING (18 sequences)

SEQ ID NO: 1 - DNA, 22 bp, Artificial Sequence
  MMP2 Forward primer
caaggatggactcctggcacat

SEQ ID NO: 2 - DNA, 22 bp, Artificial Sequence
  MMP2 reverse primer
tactcgccatcagcgttcccat

SEQ ID NO: 3 - DNA, 20 bp, Artificial Sequence
  MMP3 forward primer
ttctgggctatacgagggca

SEQ ID NO: 4 - DNA, 20 bp, Artificial Sequence
  MMP3 reverse primer
cttcttcacggttgcaggga

SEQ ID NO: 5 - DNA, 22 bp, Artificial Sequence
  MMP9 forward primer
gctgactacgataaggacggca

SEQ ID NO: 6 - DNA, 22 bp, Artificial Sequence
  MMP9 reverse primer
tagtggtgcaggcagagtagga

SEQ ID NO: 7 - DNA, 22 bp, Artificial Sequence
  TIMP1 forward primer
tcttggttccctggcgtactct

SEQ ID NO: 8 - DNA, 23 bp, Artificial Sequence
  TIMP1 reverse primer
gtgagtgtcactctccagtttgc

SEQ ID NO: 9 - DNA, 22 bp, Artificial Sequence
  TIMP2 forward primer
agccaaagcagtgagcgagaag

SEQ ID NO: 10 - DNA, 23 bp, Artificial Sequence
  TIMP2 reverse primer
gccgtgtagataaactcgatgtc

SEQ ID NO: 11 - DNA, 22 bp, Artificial Sequence
  COL1a1 forward primer
cctcagggtattgctggacaac

SEQ ID NO: 12 - DNA, 22 bp, Artificial Sequence
  COL1a1 reverse primer
cagaaggaccttgtttgccagg

SEQ ID NO: 13 - DNA, 20 bp, Artificial Sequence
  HYAL forward primer
aagtaccaaggaatcatgcc

SEQ ID NO: 14 - DNA, 20 bp, Artificial Sequence
  HYAL reverse primer
ctcaggataacttggatggc

SEQ ID NO: 15 - DNA, 20 bp, Artificial Sequence
  NF-kappa B forward primer
ttgtgccaagagtgatgacg

SEQ ID NO: 16 - DNA, 20 bp, Artificial Sequence
  NF-kappa B reverse primer
ctgaaatcccatgtcctgct

SEQ ID NO: 17 - DNA, 23 bp, Artificial Sequence
  GADPH forward primer
catcactgccacccagaagactg

SEQ ID NO: 18 - DNA, 23 bp, Artificial Sequence
  GADPH reverse primer
atgccagtgagcttcccgttcag